European Patent Application EP 4 375 299 A1, published May 29, 2024. Title: 一种B7-H3抗体及其应用. Applicant: 广州爱思迈生物医药科技有限公司. The sequence listing filed with the application follows.

SEQUENCE LISTING (51 sequences)

SEQ ID NO: 1 - protein, 124 aa, synthetic construct
  source 1..124: organism (original language) = 合成构建体
QVQLVQSGAEVKKPGSSVKVSCKASGGTFSNYAINWVRQAPGQGLEWMGGIIPLFGTANYAQKFQGRVTITADESTSTAYMELSSLRSDDTAVYYCARDQVVATSGVNFGMDVWGQGTTVTVSS

SEQ ID NO: 2 - protein, 25 aa, synthetic construct [sequence omitted]

SEQ ID NO: 3 - protein, 17 aa, synthetic construct
  source 1..17: organism (original language) = 合成构建体
INWVRQAPGQGLEWMGG

SEQ ID NO: 4 - protein, 38 aa, synthetic construct
  source 1..38: organism (original language) = 合成构建体
NYAQKFQGRVTITADESTSTAYMELSSLRSDDTAVYYC

SEQ ID NO: 5 - protein, 11 aa, synthetic construct
  source 1..11: organism (original language) = 合成构建体
WGQGTTVTVSS

SEQ ID NO: 6 - protein, 8 aa, synthetic construct
  source 1..8: organism (original language) = 合成构建体
GGTFSNYA

SEQ ID NO: 7 - protein, 8 aa, synthetic construct
  source 1..8: organism (original language) = 合成构建体
IIPLFGTA

SEQ ID NO: 8 - protein, 17 aa, synthetic construct
  source 1..17: organism (original language) = 合成构建体
ARDQVVATSGVNFGMDV

SEQ ID NO: 9 - protein, 109 aa, synthetic construct
  source 1..109: organism (original language) = 合成构建体
DIQMTQEPSLTTSPGGTVTLTCRSSTGAVTTSNYANWVQEKPGQAPRGLIGGTNKRAPGTPARFSGSLIGGKAALTITGVQPEDEAIYFCALWYSNLWVFGGGTKLEIK

SEQ ID NO: 10 - protein, 25 aa, synthetic construct
  source 1..25: organism (original language) = 合成构建体
DIQMTQEPSLTTSPGGTVTLTCRSS

SEQ ID NO: 11 - protein, 17 aa, synthetic construct
  source 1..17: organism (original language) = 合成构建体
ANWVQEKPGQAPRGLIG

SEQ ID NO: 12 - protein, 36 aa, synthetic construct
  source 1..36: organism (original language) = 合成构建体
KRAPGTPARFSGSLIGGKAALTITGVQPEDEAIYFC

SEQ ID NO: 13 - protein, 10 aa, synthetic construct
  source 1..10: organism (original language) = 合成构建体
FGGGTKLEIK

SEQ ID NO: 14 - protein, 9 aa, synthetic construct
  source 1..9: organism (original language) = 合成构建体
TGAVTTSNY

SEQ ID NO: 15 - skipped

SEQ ID NO: 16 - protein, 9 aa, synthetic construct
  source 1..9: organism (original language) = 合成构建体
ALWYSNLWV

SEQ ID NO: 17 - protein, 8 aa, synthetic construct
  source 1..8: organism (original language) = 合成构建体
GGTLRPVL

SEQ ID NO: 18 - protein, 8 aa, synthetic construct
  source 1..8: organism (original language) = 合成构建体
GGTSGVAL

SEQ ID NO: 19 - protein, 8 aa, synthetic construct
  source 1..8: organism (original language) = 合成构建体
GGTRPAAL

SEQ ID NO: 20 - protein, 8 aa, synthetic construct
  source 1..8: organism (original language) = 合成构建体
GGTVRPAL

SEQ ID NO: 21 - protein, 8 aa, synthetic construct
  source 1..8: organism (original language) = 合成构建体
GGTGGIYL

SEQ ID NO: 22 - protein, 8 aa, synthetic construct
  source 1..8: organism (original language) = 合成构建体
GGTGGAYL

SEQ ID NO: 23 - protein, 8 aa, synthetic construct
  source 1..8: organism (original language) = 合成构建体
GGTSRPVL

SEQ ID NO: 24 - protein, 8 aa, synthetic construct
  source 1..8: organism (original language) = 合成构建体
GGTRPPAL

SEQ ID NO: 25 - protein, 8 aa, synthetic construct
  source 1..8: organism (original language) = 合成构建体
GGTTGRYL

SEQ ID NO: 26 - protein, 8 aa, synthetic construct
  source 1..8: organism (original language) = 合成构建体
IIPGFYSL

SEQ ID NO: 27 - protein, 8 aa, synthetic construct
  source 1..8: organism (original language) = 合成构建体
IIPMWQSV

SEQ ID NO: 28 - protein, 8 aa, synthetic construct
  source 1..8: organism (original language) = 合成构建体
IIPLFRSS

SEQ ID NO: 29 - protein, 8 aa, synthetic construct
  source 1..8: organism (original language) = 合成构建体
IIPRFGGV

SEQ ID NO: 30 - protein, 8 aa, synthetic construct
  source 1..8: organism (original language) = 合成构建体
IIPNFESV

SEQ ID NO: 31 - protein, 8 aa, synthetic construct
  source 1..8: organism (original language) = 合成构建体
IIPKFRSQ

SEQ ID NO: 32 - protein, 8 aa, synthetic construct
  source 1..8: organism (original language) = 合成构建体
IIPVFRSV

SEQ ID NO: 33 - protein, 8 aa, synthetic construct
  source 1..8: organism (original language) = 合成构建体
IIPGFDAV

SEQ ID NO: 34 - protein, 8 aa, synthetic construct
  source 1..8: organism (original language) = 合成构建体
IIPDFNSA

SEQ ID NO: 35 - protein, 8 aa, synthetic construct
  source 1..8: organism (original language) = 合成构建体
IIPRFASR

SEQ ID NO: 36 - protein, 8 aa, synthetic construct
  source 1..8: organism (original language) = 合成构建体
IIPNFHSS

SEQ ID NO: 37 - protein, 8 aa, synthetic construct
  source 1..8: organism (original language) = 合成构建体
IIPNFYSV

SEQ ID NO: 38 - protein, 17 aa, synthetic construct
  source 1..17: organism (original language) = 合成构建体
ARDRFTPRSGVNFGMDV

SEQ ID NO: 39 - protein, 17 aa, synthetic construct
  source 1..17: organism (original language) = 合成构建体
ARDREARESGVNFGMDV

SEQ ID NO: 40 - protein, 17 aa, synthetic construct
  source 1..17: organism (original language) = 合成构建体
ARDFDAPGSGVNFGMDV

SEQ ID NO: 41 - protein, 17 aa, synthetic construct
  source 1..17: organism (original language) = 合成构建体
ARDVVVPRSGVNFGMDV

SEQ ID NO: 42 - protein, 17 aa, synthetic construct
  source 1..17: organism (original language) = 合成构建体
ARDIEVMASGVNFGMDV

SEQ ID NO: 43 - protein, 17 aa, synthetic construct
  source 1..17: organism (original language) = 合成构建体
ARDQVVPLSGVNFGMDV

SEQ ID NO: 44 - protein, 17 aa, synthetic construct
  source 1..17: organism (original language) = 合成构建体
ARDVNNPGSGVNFGMDV

SEQ ID NO: 45 - protein, 17 aa, synthetic construct
  source 1..17: organism (original language) = 合成构建体
ARDVEVFNSGVNFGMDV

SEQ ID NO: 46 - protein, 17 aa, synthetic construct
  source 1..17: organism (original language) = 合成构建体
ARDEVVVGSGVNFGMDV

SEQ ID NO: 47 - protein, 17 aa, synthetic construct
  source 1..17: organism (original language) = 合成构建体
ARDAVVPNSGVNFGMDV

SEQ ID NO: 48 - protein, 17 aa, synthetic construct
  source 1..17: organism (original language) = 合成构建体
ARDQVVPRSGVNFGMDV

SEQ ID NO: 49 - protein, 125 aa, synthetic construct
  source 1..125: organism (original language) = 合成构建体
EVQLVESGGGLVQPGGSLKLSCAASGFTFNTYAMNWVRQAPGKGLEWVARIRSKYNNYATYYADSVKDRFTISRDDSKNTAYLQMNNLKTEDTAMYYCVRHGNFGTSYVSWFAYWGQGTLVTVSS

SEQ ID NO: 50 - DNA, 327 bp, synthetic construct
  source 1..327: mol_type = other DNA; organism (original language) = 合成构建体
gatattcagatgacacaagaaccaagtctcactacaagccctggaggcaccgttacactgacctgtcgctcttccactggcgccgtgaccacttccaactatgcaaactgggtgcaggagaaacctggacaggctcctagaggtctgattggaggcactaacaagagagctccagggactcctgccaggttcagcggatctctgatcggtgggaaggcagctctgacaatcactggagtgcaacccgaggatgaggctatctacttctgtgctctctggtactcaaatctgtgggtgttcggaggtggaacaaagctggagatcaag

SEQ ID NO: 51 - DNA, 372 bp, synthetic construct
  source 1..372: mol_type = other DNA; organism (original language) = 合成构建体
caggtccagcttgtgcagtctggggctgaggtgaagaagcctgggtcctcggtgaaggtctcctgcaaggcttctggaggcaccttcagcaactatgctatcaactgggtgcgacaggcccctggacaagggcttgagtggatgggagggatcatccctctctttggtacagcaaactacgcacagaagttccagggcagagtcacgattaccgcggacgaatccacgagcacagcctacatggagctgagcagcctgagatctgacgacacggccgtgtattactgtgcgagagaccaggtagtggcaacgagtggcgtcaacttcggtatggacgtctggggccaagggaccacggtcaccgtctcctca